European Patent Application EP 4 806 994 A1, published September 16, 2026. Title: Synthetic Lipase Enzymes and Uses Thereof. Applicant: ASOCIACIÓN CENTRO DE INVESTIGACIÓN COOPERATIVA EN BIOCIENCIAS-CIC bioGUNE. The sequence listing filed with the application follows.

SEQUENCE LISTING (24 sequences)

SEQ ID NO: 1 - protein, 181 aa, Bacillus subtilis
AEHNPVVMVHGIGGASFNFAGIKSYLVSQGWSRDKLYAVDFWDKTGTNYNNGPVLSRFVQKVLDETGAKKVDIVAHSMGGANTLYYIKNLDGGNKVANVVTLGGANRLTTGKALPGTDPNQKILYTSIYSSADMIVMNYLSRLDGARNVQIHGVGHIGLLYSSQVNSLIKEGLNGGGQNTN

SEQ ID NO: 2 - protein, 181 aa, synthetic construct
AEHNPVVMVHGIGGASFNFAGIKSYLVSQGWSRDKLYAVDFWDKTGTNENNGPVLSRFVQKVLDETGAKKVDIVAHSMGGANTLYYIKNLDGGNKVANVVTLGGANRLTTGKALPGTDPNQKILYTSIYSSADMIVMNYLSRLEGARNVQIHGVGHIGLLTSSQVNDLIKEGLNGGGQNTN

SEQ ID NO: 3 - protein, 181 aa, synthetic construct
AEHNPVVMVHGIGGASFNFAGIKSYLVSQGWSRDKLYAVDFWDKTGTNENNGPVLSRFVQKVLDETGAKKVDIVAHSMGGANTLYYIKNLDGGNKVANVVTLGGANRLTTGKALPGTDPNQKILYTSIYSSADMIVMNYLSRLSGARNVQIHGVGHIGLLTSSQVNDLIKEGLNGGGQNTN

SEQ ID NO: 4 - protein, 181 aa, synthetic construct
AEHNPVVMVHGIGGASFNFAGIKSYLVSQGWSRDKLYAVDFPDKTGTNENNGPVLSRFVQKVLDETGAKKVDIVAHSMGGANTLYYIKNLDGGNKVANVVTLGGANRLTTGKALPGTDPNQKILYTSIYSSADTIVPNYLSRLEGARNVQIHGVGHIGLLTSSQVNDLIKEGLNGGGQNTN

SEQ ID NO: 5 - protein, 181 aa, synthetic construct
AEHNPVVMVHGIGGASFNFAGIKSYLVSQGWSRDKLYAVDFWDKTGTNENNGPVLSRFVQKVLDETGAKKVDIVAHSMGGANTLYYIKNLDGGNKVANVVTLGGANRLTTGKALPGTDPNQKILYTSIYSSADTIVPNYLSRLEGARNVQIHGVGHIGLLTSSQVNDLIKEGLNGGGQNTN

SEQ ID NO: 6 - protein, 181 aa, synthetic construct
AEHNPVVMVHGIGGASFNFDGIKDYLVSQGWSRDKLYAVDFPDKTGTNENNGPVLSAFVQKVLDETGAKKVDIVAHSMGGANTLYYIKNLDGGNKVANVVTLGGANRLTTGTALPGTDPNQKILYTSIYSSADMIVMNYLSRLEGARNVQIHGVGHIGLLTSSQVNDLIKEGLNGGGQNTN

SEQ ID NO: 7 - protein, 181 aa, synthetic construct
AEHNPVVMVHGIGGASFNFDGIKDYLVSQGWSRDKLYAVDFWDKTGTNENNGPVLSAFVQKVLDETGAKKVDIVAHSMGGANTLYYIKNLDGGNKVANVVTLGGANRLTTGTALPGTDPNQKILYTSIYSSADMIVPNYLSRLEGARNVQIHGVGHIGLLTSSQVNDLIKEGLNGGGQNTN

SEQ ID NO: 8 - protein, 181 aa, synthetic construct
AEHNPVVMVHGIGGASFNFDGIKDYLVSQGWSRDKLYAVDFPDKTGTNENNGPVLSAFVQKVLDETGAKKVDIVAHSMGGANTLYYIKNLDGGNKVANVVTLGGANRLTTGTALPGTDPNQKILYTSIYSSADMIVPNYLSRLEGARNVQIHGVGHIGLLTSSQVNDLIKEGLNGGGQNTN

SEQ ID NO: 9 - protein, 181 aa, synthetic construct
AEHNPVVMVHGIGGASFNFDGIKDYLVSQGWSRDKLYAVDFWDKTGTNENNGPVLSAFVQKVLDETGAKKVDIVAHSMGGANTLYYIKNLDGGNKVANVVTLGGANRLTTGTALPGTDPNQKILYTSIYSSADTIVPNYLSRLEGARNVQIHGVGHIGLLTSSQVNDLIKEGLNGGGQNTN

SEQ ID NO: 10 - protein, 181 aa, synthetic construct
AEHNPVVMVHGIGGASFNFDGIKDYLVSQGWSRDKLYAVDFPDKTGTNENNGPVLSAFVQKVLDETGAKKVDIVAHSMGGANTLYYIKNLDGGNKVANVVTLGGANRLTTGTALPGTDPNQKILYTSIYSSADTIVPNYLSRLEGARNVQIHGVGHIGLLTSSQVNDLIKEGLNGGGQNTN

SEQ ID NO: 11 - protein, 181 aa, synthetic construct
AEHNPVVMVHGIGGASSNFDGIKDYLVSQGWSRDKLYAVDFPDKTGTNENNGPVLSAFVDKVLDETGAKKVDIVAHSMGGANTLYYIKNLDGGDKVANVVTLGGANRLTTGTALPGTDPNQKILYTSIYSSADTIVPNYLSRLEGAKNVQISGVGHIGLLTSSQVFDLIKEGLNGGGQNTN

SEQ ID NO: 12 - protein, 181 aa, synthetic construct
AEHNPVVMVHGIGGAASNFDGIKDYLVSQGWSRDKLYAVDFPDKTGTNENNGPVLSAFVDKVLDETGAKKVDIVAHSMGGANTLYYIKNLDGGDKVANVVTLGGANRLTTGTALPGTDPNQKILYTSIYSSADTIVPNYLSRLEGAKNVQISGVGHIGLLTSSQVFDLVKEGLDGGGQNTN

SEQ ID NO: 13 - protein, 181 aa, synthetic construct
AEHNPVVMVHGVGGAASNFDAIKDYLVSQGWDRDKLYAVDFPDKTGTNEKNGPVLSAFVDKVLDETGAKKVDIVAHSMGGANTLYYIKNLDGGDKVANVVTLGGANRLTTGTADPGTDPNQKILYTSIYSSADTIVPNSLSRLEGAKNVLISGVDHIGLLTSSEVFDLVKEGLDGGGQNTN

SEQ ID NO: 14 - protein, 181 aa, synthetic construct
AEHNPVVMVHGVGGAASNFDAIKAYLVSKGWDASKLYAVDFPDKTGANEKNGPVLSAFVDKVLKETGADKVDIVAHSMGGANTLYYIKNLDGGDKVANVVTLGGANALTTTTADPGTDPNQKILYTSIYSTADTIVPNSLSWLSGAKNVLISGVDHYGLLTSSEVFDLVKEGLDGGGQNTN

SEQ ID NO: 15 - protein, 181 aa, synthetic construct
AEHNPVVMVHGIGGASSNFDAIKDYLVSQGWDRSKLYAVDFPDKTGTNENNGPVLSAFVDKVLKETGAKKVDIVAHSMGGANTLYYIKNLDGGDKVANVVTLGGANRLTTGTALPGTDPNQKILYTSIYSSADTIVPNSLSYLEGAKNVLISGVGHIGLLTSSQVFDLIKEGLNGGGQNTN

SEQ ID NO: 16 - protein, 6 aa, synthetic construct
HHHHHH

SEQ ID NO: 17 - protein, 5 aa, synthetic construct
GGGGS

SEQ ID NO: 18 - protein, 8 aa, synthetic construct
HHHHHHGS

SEQ ID NO: 19 - protein, 181 aa, synthetic construct
AEHNPVVMVHGIGGASFNFANIKDYLVSQGWSRDKLYAVDFWDKTGTNEKNGPQLSKFVQKVLDETGAKKVDIVAHSMGGANTLYYIKNLDGGNKVANVVTLGGANRLTTGKALPGTDPNQKILYTSIYSSADMIVMNELSRLDGARNVQIHGVGHIGLLYSSEVNSLIKEGLNGGGQNTN

SEQ ID NO: 20 - protein, 181 aa, synthetic construct
AEHNPVVMVHGIGGASFNFDYIKDYLVSKGWSRDKLYAVDFWDKTGTNEKNGPVLSKFVNKVLKETGAKKVDIVAHSMGGANTLYYIKNLDGGNKVANVVTLGGANRLTTGKALPGTDPNQKILYTSIYSSADMIVMNYLSRLDGARNVQIHGVGHIGLLYSSEVNSLIKEGLNGGGQNTN

SEQ ID NO: 21 - protein, 181 aa, synthetic construct
AEHNPVVMVHGIGGASFNFDNIKDYLVSQGWSRDKLYAVDFWDKTGTNEKNGPQLEKFVQKVLKETGAKKVDIVAHSMGGANTLYYIKNLDGGNKVANVVTLGGANRLTTGKALPGTDPNQKILYTSIYSSADMIVMNELSRLDGARNVQIHGVGHIGLLYSSEVNELIKEGLNGGGQNTN

SEQ ID NO: 22 - protein, 181 aa, synthetic construct
ASHNPVVMVHGIGGASFNFDGIKSYLVSQGWDEDKLYAVDFSDKTGSNEKNGPELEKFVQKVLDETGAEKVDIVAHSMGGANTLYYIKNLDGGDKVANVVTLGGANRLTTGKALPGTDPNQKILYTSIYSSADMIVMNYLSRLDGARNVQISGVGHIGLLYSSEVNDLIKEGLNGGGQNTN

SEQ ID NO: 23 - protein, 181 aa, synthetic construct
AEHNPVVMVHGIGGASFNFDYIKDYLVSKGWSRDKLYAVDFWDKTGTQEKNGPQLEKFVNSVLKETGAKKVDIVAHSMGGANTLYYIKNLDGGNKVANVVTLGGANRLTTGKALPGTDPNQKILYTSIYSSADMIVMNELSRLDGARNVQIHGVGHIGLLYSEEVAEYIYEGLNGGGQNTN

SEQ ID NO: 24 - protein, 181 aa, synthetic construct
ASHNPVVMVHGIGGSSDNFDNIKSYLVSQGWDEDKLYAVDFSDKTGSNEKNGPELEKFVQKVLKETGAEKVDIVAHSMGGANTLYYIKNLDGGDKVRNVVTLGGANRLTTSEALPGTDPNQKILYTSIYSSADMIVMNELSELKGARNVQISGVGHIGLLNSSEVNDLIKEGLNGGGENTN